European Patent Specification EP 4 551 718 B1, published June 24, 2026. Title: PCR-FREE LIBRARY PREPARATION USING DOUBLE-STRANDED SPLINT ADAPTORS AND METHODS OF USE. Applicant: ELEMENT BIOSCIENCES, INC. Application US. The sequence listing filed with the application follows.

SEQUENCE LISTING (64 sequences)

SEQ ID NO: 1 - DNA, 35 bp, synthetic construct
  source 1..35: mol_type = other DNA
cgtgctggattggctcaccagacaccttccgacat

SEQ ID NO: 2 - DNA, 33 bp, synthetic construct
  source 1..33: mol_type = other DNA
acactctttccctacacgacgctcttccgatct

SEQ ID NO: 3 - DNA, 33 bp, synthetic construct
  source 1..33: mol_type = other DNA
tcgtcggcagcgtcagatgtgtataagagacag

SEQ ID NO: 4 - DNA, 35 bp, synthetic construct
  source 1..35: mol_type = other DNA
atgtcggaaggtgtgcaggctaccgcttgtcaact

SEQ ID NO: 5 - DNA, 34 bp, synthetic construct
  source 1..34: mol_type = other DNA
agatcggaagagcacacgtctgaactccagtcac

SEQ ID NO: 6 - DNA, 34 bp, synthetic construct
  source 1..34: mol_type = other DNA
ctgtctcttatacacatctccgagcccacgagac

SEQ ID NO: 7 - DNA, 35 bp, synthetic construct
  source 1..35: mol_type = other DNA
atgtcggaaggtgtctggtgagccaatccagcacg

SEQ ID NO: 8 - DNA, 18 bp, synthetic construct
  source 1..18: mol_type = other DNA
gtgagccaatccagcacg

SEQ ID NO: 9 - DNA, 33 bp, synthetic construct
  source 1..33: mol_type = other DNA
agatcggaagagcgtcgtgtagggaaagagtgt

SEQ ID NO: 10 - DNA, 33 bp, synthetic construct
  source 1..33: mol_type = other DNA
ctgtctcttatacacatctgacgctgccgacga

SEQ ID NO: 11 - DNA, 35 bp, synthetic construct; identical to SEQ ID NO: 4
  source 1..35: mol_type = other DNA

SEQ ID NO: 12 - DNA, 18 bp, synthetic construct
  source 1..18: mol_type = other DNA
agttgacaagcggtagcc

SEQ ID NO: 13 - DNA, 34 bp, synthetic construct
  source 1..34: mol_type = other DNA
gtgactggagttcagacgtgtgctcttccgatct

SEQ ID NO: 14 - DNA, 34 bp, synthetic construct
  source 1..34: mol_type = other DNA
gtctcgtgggctcggagatgtgtataagagacag

SEQ ID NO: 15-17 - skipped (3 entries)

SEQ ID NO: 18 - DNA, 23 bp, synthetic construct
  source 1..23: mol_type = other DNA
ctagtccactccgacgctgctga

SEQ ID NO: 19 - DNA, 22 bp, synthetic construct
  source 1..22: mol_type = other DNA
taatgtacctagtccactccga

SEQ ID NO: 20 - DNA, 31 bp, synthetic construct
  source 1..31: mol_type = other DNA
taatgtacctagtccactccgacgctgctga

SEQ ID NO: 21 - DNA, 15 bp, synthetic construct
  source 1..15: mol_type = other DNA
ctccgacgctgctga

SEQ ID NO: 22 - DNA, 24 bp, synthetic construct
  source 1..24: mol_type = other DNA
gttcgtcttctgccgtatgctcta

SEQ ID NO: 23 - DNA, 25 bp, synthetic construct
  source 1..25: mol_type = other DNA
tgggactttcatgcacgtaatgtac

SEQ ID NO: 24 - DNA, 17 bp, synthetic construct
  source 1..17: mol_type = other DNA
tgggactttcatgcacg

SEQ ID NO: 25 - DNA, 33 bp, synthetic construct
  source 1..33: mol_type = other DNA
tgggactttcatgcacgtaatgtacctagtcca

SEQ ID NO: 26 - DNA, 24 bp, synthetic construct
  source 1..24: mol_type = other DNA
ctagagccaccagcggcatagtaa

SEQ ID NO: 27-33 - skipped (7 entries)

SEQ ID NO: 34 - DNA, 23 bp, synthetic construct
  source 1..23: mol_type = other DNA
gatcaggtgaggctgcgacgact

SEQ ID NO: 35 - DNA, 22 bp, synthetic construct
  source 1..22: mol_type = other DNA
attacatggatcaggtgaggct

SEQ ID NO: 36 - DNA, 15 bp, synthetic construct
  source 1..15: mol_type = other DNA
gaggctgcgacgact

SEQ ID NO: 37 - DNA, 21 bp, synthetic construct
  source 1..21: mol_type = other DNA
caagcagaagacggcatacga

SEQ ID NO: 38 - DNA, 24 bp, synthetic construct
  source 1..24: mol_type = other DNA
caagcagaagacggcatacgagat

SEQ ID NO: 39 - DNA, 25 bp, synthetic construct
  source 1..25: mol_type = other DNA
catgtaatgcacgtactttcagggt

SEQ ID NO: 40 - DNA, 33 bp, synthetic construct
  source 1..33: mol_type = other DNA
acctgatccatgtaatgcacgtactttcagggt

SEQ ID NO: 41 - DNA, 20 bp, synthetic construct
  source 1..20: mol_type = other DNA
aatgatacggcgaccaccga

SEQ ID NO: 42 - DNA, 24 bp, synthetic construct
  source 1..24: mol_type = other DNA
aatgatacggcgaccaccgagatc

SEQ ID NO: 43 - DNA, 30 bp, synthetic construct
  source 1..30: mol_type = other DNA
atgtcggaaggtgtgcaggctaccgcttgt

SEQ ID NO: 44 - DNA, 25 bp, synthetic construct
  source 1..25: mol_type = other DNA
atgtcggaaggtgtgcaggctaccg

SEQ ID NO: 45 - DNA, 25 bp, synthetic construct
  source 1..25: mol_type = other DNA
taatgtacctagtccactccgacgc

SEQ ID NO: 46 - DNA, 27 bp, synthetic construct
  source 1..27: mol_type = other DNA
cgtactaatgtacctagtccactccga

SEQ ID NO: 47 - DNA, 25 bp, synthetic construct
  source 1..25: mol_type = other DNA
tgggactttcatgcacgtaatgtac

SEQ ID NO: 48 - skipped

SEQ ID NO: 49 - DNA, 22 bp, synthetic construct
  source 1..22: mol_type = other DNA
tgggactttcatgcacgattgc

SEQ ID NO: 50 - DNA, 25 bp, synthetic construct
  source 1..25: mol_type = other DNA
attacatggatcaggtgaggctgcg

SEQ ID NO: 51 - DNA, 35 bp, synthetic construct; identical to SEQ ID NO: 1
  source 1..35: mol_type = other DNA

SEQ ID NO: 52 - DNA, 35 bp, synthetic construct
  source 1..35: mol_type = other DNA
agttgacaagcggtagcctgcacaccttccgacat

SEQ ID NO: 53 - DNA, 30 bp, synthetic construct
  source 1..30: mol_type = other DNA
acaagcggtagcctgcacaccttccgacat

SEQ ID NO: 54 - DNA, 22 bp, synthetic construct
  source 1..22: mol_type = other DNA
agcctcacctgatccatgtaat

SEQ ID NO: 55 - DNA, 27 bp, synthetic construct
  source 1..27: mol_type = other DNA
agcctcacctgatccatgtaatcatgc

SEQ ID NO: 56 - DNA, 23 bp, synthetic construct
  source 1..23: mol_type = other DNA
agtcgtcgcagcctcacctgatc

SEQ ID NO: 57 - DNA, 31 bp, synthetic construct
  source 1..31: mol_type = other DNA
agtcgtcgcagcctcacctgatccatgtaat

SEQ ID NO: 58 - DNA, 36 bp, synthetic construct
  source 1..36: mol_type = other DNA
agtcgtcgcagcctcacctgatccatgtaatcgtga

SEQ ID NO: 59 - DNA, 36 bp, synthetic construct
  source 1..36: mol_type = other DNA
agtcgtcgcagcctcacctgatccatgtaatcatgc

SEQ ID NO: 60 - DNA, 35 bp, synthetic construct; identical to SEQ ID NO: 4
  source 1..35: mol_type = other DNA

SEQ ID NO: 61 - DNA, 25 bp, synthetic construct
  source 1..25: mol_type = other DNA
accctgaaagtacgtgcattacatg

SEQ ID NO: 62 - DNA, 17 bp, synthetic construct
  source 1..17: mol_type = other DNA
accctgaaagtacgtgc

SEQ ID NO: 63 - DNA, 22 bp, synthetic construct
  source 1..22: mol_type = other DNA
accctgaaagtacgtgctaacg

SEQ ID NO: 64 - DNA, 33 bp, synthetic construct
  source 1..33: mol_type = other DNA
accctgaaagtacgtgcattacatggatcaggt